European Patent Application EP 4 600 263 A1, published August 13, 2025. Title: KERATIN YK93-9, PREPARATION METHOD THEREFOR, PHARMACEUTICAL COMPOSITION THEREOF, AND USE THEREOF. Applicant: Institute of Materia Medica Chinese Academy Of Medical Sciences. The sequence listing filed with the application follows.

SEQUENCE LISTING (2 sequences)

SEQ ID NO: 1 - protein, 593 aa, Manis pentadactyla
MSLQSKVSVRSGGSRSFSAASAITPSISRTSFTSVSRSGGGGGGFGRVSLGGVCGAGGYGSRSLYNLGGSKRISISTSGGSFRNRFGAGAGGGYGFAGGAGSGFGFGGGAGGGFGLGGGAGFGGGFGGPGFPVCPPGGIQEVTINQNLLTPLNLQIDPTIQRVRTEEREQIKTLNNKFASFIDKVRFLEQQNKVLDTKWTLLQEQGTKTVRQNLEPLFEQYINNLRRQLDSILGERGRLDSELRNMQDLVEDFKNKYEDEINKRTTAENEFVMLKKDVDAAYMNKVELEAKVDALMDEINFMKMFFEAELSQMQTHVSDTSVILSMDNNRNLDLDSIIAEVKAQYEEIANRSRTEAESWYQTKYEELQQTAGRHGDDLRNTKHEISEMNRMIQRLRAEIDNVKKQCASLQAAIADAEQRGELALKDARNKLAELEDALQKAKQDMARLLREYQELMNTKLALDVEIATYRKLLEGEECRLSGEGVGPVNISVVTNSISSSYGGGSGFGGGLSGGLGSGLGGGLGSGLGGGGGVSYYSSSSGGVGLGSGLSAGGAGFSAGSGRSLGVGLGSGGASSSSVKFVSTTSSSRKSIKS

SEQ ID NO: 2 - DNA, 1779 bp, Manis pentadactyla
  source 1..1779: mol_type = genomic DNA
atgagcctgcagagcaaagttagcgtgcgtagtggtggcagccgcagttttagcgccgccagcgccattaccccgagcattagccgcaccagctttaccagtgttagccgcagcggtggcggtggtggtggttttggccgtgtgagcctgggtggtgtgtgtggtgcaggtggctatggcagccgtagcctgtataatctgggcggcagtaaacgcattagcattagtaccagcggtggtagttttcgtaatcgctttggtgcaggtgcaggtggtggctatggttttgcaggtggcgccggtagtggctttggttttggcggtggcgccggcggtggctttggcttaggcggtggcgcgggctttggcggtggttttggtggtccgggctttccggtgtgtccgccgggtggtattcaggaagttaccattaatcagaatctgctgaccccgctgaatctgcagattgatccgaccattcagcgcgttcgcaccgaagaacgcgaacagattaagaccctgaataataagtttgcaagttttatcgacaaggtgcgctttctggaacagcagaataaggttctggataccaaatggaccctgctgcaggaacagggtaccaaaaccgtgcgccagaatctggaaccgctgtttgaacagtatattaataatctgcgtcgtcagctggatagcattctgggcgaacgtggccgtctggatagtgaactgcgcaatatgcaggatctggtggaagattttaaaaataagtacgaagacgagatcaacaaacgcaccaccgcagaaaatgaatttgttatgctgaaaaaggacgtggatgccgcctatatgaataaggtggaactggaagccaaagttgatgccctgatggatgaaattaattttatgaaaatgttcttcgaggcggaactgagtcagatgcagacccatgtgagcgataccagtgttattctgagtatggataataatcgcaatctggatctggatagtattattgcagaagttaaagcccagtatgaagaaattgcaaatcgcagtcgtaccgaagccgaaagttggtatcagaccaaatatgaagaactgcagcagaccgccggtcgtcatggcgatgatctgcgtaataccaaacatgaaattagtgaaatgaaccgtatgattcagcgcctgcgcgcagaaattgataatgttaaaaaacagtgcgcaagtctgcaggcagcaattgccgatgccgaacagcgtggcgaactggccctgaaagatgcccgtaataagctggccgaactggaagatgccctgcagaaagccaaacaggatatggcacgcctgctgcgcgaatatcaggaactgatgaataccaaactggccctggatgttgaaattgcaacctatcgtaaactgctggaaggtgaagaatgccgcctgagcggcgaaggtgtgggtccggtgaatattagcgttgttaccaatagcattagtagcagttatggcggcggcagtggctttggcggcggtttaagcggtggtctgggtagcggtctgggcggcggtctgggttcaggcctgggtggtggcggcggtgtgagttattatagtagcagcagtggcggtgtgggcctgggtagtggcctgagcgcaggtggcgcaggctttagcgccggcagtggccgtagcctgggcgttggtctgggcagtggtggcgccagcagtagcagcgtgaaatttgtgagtaccaccagcagtagtcgcaaaagcattaagagt